European Patent Application EP 4 350 007 A1, published April 10, 2024. Title: SEQUENCING METHOD. Applicant: Shenzhen GeneMind Biosciences Co., Ltd. The sequence listing filed with the application follows.

SEQUENCE LISTING (13 sequences)

SEQ ID NO: 1 - DNA, 26 bp, Artificial Sequence
  adapter or primer
  misc_feature (1)..(26): i5 index sequencing primer
gatacggcgaccaccgagatctacac

SEQ ID NO: 2 - DNA, 33 bp, Artificial Sequence
  adapter or primer
  misc_feature (1)..(33): i7 index sequencing primer
gatcggaagagcacacgtctgaactccagtcac

SEQ ID NO: 3 - DNA, 33 bp, Artificial Sequence
  adapter or primer
  misc_feature (1)..(33): insert fragment or sequencing primer
acactctttccctacacgacgctcttccgatct

SEQ ID NO: 4 - DNA, 34 bp, Artificial Sequence
  adapter or primer
  misc_feature (1)..(34): solid-phase primer
ttttttttttcaagcagaagacggcatacgagat

SEQ ID NO: 5 - DNA, 39 bp, Artificial Sequence
  adapter or primer
  misc_feature (1)..(39): solid-phase primer
  misc_feature (10)..(10): 2-deoxyuridin
tttttttttuaatgatacggcgaccaccgagatctacac

SEQ ID NO: 6 - DNA, 39 bp, Artificial Sequence
  adapter or primer
  misc_feature (1)..(39): solid-phase primer
  misc_feature (13)..(13): 2-deoxyuridin
ttttttttttaaugatacggcgaccaccgagatctacac

SEQ ID NO: 7 - DNA, 39 bp, Artificial Sequence
  adapter or primer
  misc_feature (1)..(39): solid-phase primer
  misc_feature (16)..(16): 2-deoxyuridin
ttttttttttaatgauacggcgaccaccgagatctacac

SEQ ID NO: 8 - DNA, 39 bp, Artificial Sequence
  adapter or primer
  misc_feature (1)..(39): solid-phase primer
  misc_feature (33)..(33): 2-deoxyuridin
ttttttttttaatgatacggcgaccaccgagauctacac

SEQ ID NO: 9 - DNA, 31 bp, Artificial Sequence
  adapter or primer
  misc_feature (1)..(31): adapter
  modified_base (31)..(31): ligated with ddNTP、amino or PEG
gatcggaagagcacacgtctgaactccagtc

SEQ ID NO: 10 - DNA, 33 bp, Artificial Sequence; identical to SEQ ID NO: 3
  adapter or primer
  misc_feature (1)..(33): adapter

SEQ ID NO: 11 - DNA, 65 bp, Artificial Sequence
  adapter or primer
  misc_feature (1)..(65): primer
  misc_feature (25)..(32): label，n is a or g or c or t/u
caagcagaagacggcatacgagatnnnnnnnngtgactggagttcagacgtgtgctcttccgatc

SEQ ID NO: 12 - DNA, 58 bp, Artificial Sequence
  adapter or primer
  misc_feature (1)..(58): primer
aatgatacggcgaccaccgagatctacactctttccctacacgacgctcttccgatct

SEQ ID NO: 13 - DNA, 70 bp, Artificial Sequence
  adapter or primer
  misc_feature (1)..(70): primer
  misc_feature (30)..(37): label，n is a or g or c or t/u
aatgatacggcgaccaccgagatctacacnnnnnnnnacactctttccctacacgacgctcttccgatct